European Patent Application EP 4 563 597 A1, published June 4, 2025. Title: Anti-ROR1 Antibody and Use Thereof. Applicant: AIMED BIO INC. The sequence listing filed with the application follows.

SEQUENCE LISTING (200 sequences)

SEQ ID NO: 1 - protein, 5 aa, synthetic construct
  REGION 1..5: note = Synthetic Sequence
NYDMS

SEQ ID NO: 2 - protein, 5 aa, synthetic construct
  REGION 1..5: note = Synthetic Sequence
DYSMS

SEQ ID NO: 3 - protein, 5 aa, synthetic construct
  REGION 1..5: note = Synthetic Sequence
SYAMS

SEQ ID NO: 4 - protein, 5 aa, synthetic construct
  REGION 1..5: note = Synthetic Sequence
DYAMA

SEQ ID NO: 5 - protein, 5 aa, synthetic construct
  REGION 1..5: note = Synthetic Sequence
NYSMS

SEQ ID NO: 6 - protein, 5 aa, synthetic construct
  REGION 1..5: note = Synthetic Sequence
GYSMS

SEQ ID NO: 7 - protein, 5 aa, synthetic construct
  REGION 1..5: note = Synthetic Sequence
NYAMS

SEQ ID NO: 8 - protein, 5 aa, synthetic construct
  REGION 1..5: note = Synthetic Sequence
SYDMS

SEQ ID NO: 9 - protein, 5 aa, synthetic construct
  REGION 1..5: note = Synthetic Sequence
SYSMS

SEQ ID NO: 10 - protein, 5 aa, synthetic construct
  REGION 1..5: note = Synthetic Sequence
DYAMS

SEQ ID NO: 11 - protein, 5 aa, synthetic construct
  REGION 1..5: note = Synthetic Sequence
GYAMS

SEQ ID NO: 12 - protein, 5 aa, synthetic construct
  REGION 1..5: note = Synthetic Sequence
SYAKH

SEQ ID NO: 13 - protein, 5 aa, synthetic construct
  REGION 1..5: note = Synthetic Sequence
GYYMS

SEQ ID NO: 14 - protein, 5 aa, synthetic construct
  REGION 1..5: note = Synthetic Sequence
GYDMS

SEQ ID NO: 15 - protein, 5 aa, synthetic construct
  REGION 1..5: note = Synthetic Sequence
DYYMS

SEQ ID NO: 16 - protein, 5 aa, synthetic construct
  REGION 1..5: note = Synthetic Sequence
NYAMH

SEQ ID NO: 17 - protein, 17 aa, synthetic construct
  REGION 1..17: note = Synthetic Sequence
GIYSGNSNTYYADSVKG

SEQ ID NO: 18 - protein, 17 aa, synthetic construct
  REGION 1..17: note = Synthetic Sequence
GISHNGGSTYYADSVKG

SEQ ID NO: 19 - protein, 17 aa, synthetic construct
  REGION 1..17: note = Synthetic Sequence
GISPGGSSKYYADSVKG

SEQ ID NO: 20 - protein, 17 aa, synthetic construct
  REGION 1..17: note = Synthetic Sequence
IIYPGDSETIYSPSFEG

SEQ ID NO: 21 - protein, 17 aa, synthetic construct
  REGION 1..17: note = Synthetic Sequence
AISHGSGSIYYADSVKG

SEQ ID NO: 22 - protein, 16 aa, synthetic construct
  REGION 1..16: note = Synthetic Sequence
GISYGGSSIYADSVKG

SEQ ID NO: 23 - protein, 17 aa, synthetic construct
  REGION 1..17: note = Synthetic Sequence
GISPNGSSIYYADSVKG

SEQ ID NO: 24 - protein, 17 aa, synthetic construct
  REGION 1..17: note = Synthetic Sequence
GISPDGGSIYYADSVKG

SEQ ID NO: 25 - protein, 17 aa, synthetic construct
  REGION 1..17: note = Synthetic Sequence
GISYGGSSISYADSVKG

SEQ ID NO: 26 - protein, 17 aa, synthetic construct
  REGION 1..17: note = Synthetic Sequence
WISHGGGSIYYADSVKG

SEQ ID NO: 27 - protein, 16 aa, synthetic construct
  REGION 1..16: note = Synthetic Sequence
ISPGDSNKYYADSVKG

SEQ ID NO: 28 - protein, 17 aa, synthetic construct
  REGION 1..17: note = Synthetic Sequence
GISPGGGSIYYADSVKG

SEQ ID NO: 29 - protein, 17 aa, synthetic construct
  REGION 1..17: note = Synthetic Sequence
AISHGGSSKYYADSVKG

SEQ ID NO: 30 - protein, 17 aa, synthetic construct
  REGION 1..17: note = Synthetic Sequence
VISPGSGSKYYADSVRG

SEQ ID NO: 31 - protein, 15 aa, synthetic construct
  REGION 1..15: note = Synthetic Sequence
IYTSGSTNYNPSLKS

SEQ ID NO: 32 - protein, 17 aa, synthetic construct
  REGION 1..17: note = Synthetic Sequence
VISHDGSSTYYADSVKG

SEQ ID NO: 33 - protein, 17 aa, synthetic construct
  REGION 1..17: note = Synthetic Sequence
WISPGGGNIYYADSVKG

SEQ ID NO: 34 - protein, 17 aa, synthetic construct
  REGION 1..17: note = Synthetic Sequence
SISSNGGSTYYADSVKG

SEQ ID NO: 35 - protein, 17 aa, synthetic construct
  REGION 1..17: note = Synthetic Sequence
GISHDGRSKYYADSVKG

SEQ ID NO: 36 - protein, 17 aa, synthetic construct
  REGION 1..17: note = Synthetic Sequence
LISPGSDSKYYADSVKG

SEQ ID NO: 37 - protein, 17 aa, synthetic construct
  REGION 1..17: note = Synthetic Sequence
AISYDNGNTYYADSVKG

SEQ ID NO: 38 - protein, 17 aa, synthetic construct
  REGION 1..17: note = Synthetic Sequence
WISPGGGNTYYADSVKG

SEQ ID NO: 39 - protein, 17 aa, synthetic construct
  REGION 1..17: note = Synthetic Sequence
VISSDGGSIYYADSVKG

SEQ ID NO: 40 - protein, 17 aa, synthetic construct
  REGION 1..17: note = Synthetic Sequence
WISPGGSSIYYADSVKG

SEQ ID NO: 41 - protein, 17 aa, synthetic construct
  REGION 1..17: note = Synthetic Sequence
SIIYPDDDTRYNPSFRG

SEQ ID NO: 42 - protein, 12 aa, synthetic construct
  REGION 1..12: note = Synthetic Sequence
DLQYTEWAGFDY

SEQ ID NO: 43 - protein, 18 aa, synthetic construct
  REGION 1..18: note = Synthetic Sequence
DVSRWSKTRWSYDNAMDV

SEQ ID NO: 44 - protein, 13 aa, synthetic construct
  REGION 1..13: note = Synthetic Sequence
RGPHRAIDTAFDY

SEQ ID NO: 45 - protein, 11 aa, synthetic construct
  REGION 1..11: note = Synthetic Sequence
RDTYWEGYFDL

SEQ ID NO: 46 - protein, 19 aa, synthetic construct
  REGION 1..19: note = Synthetic Sequence
KPISAWSHIRMSYAYGMDV

SEQ ID NO: 47 - protein, 19 aa, synthetic construct
  REGION 1..19: note = Synthetic Sequence
KPVRRWARFRLSYDDAMDV

SEQ ID NO: 48 - protein, 18 aa, synthetic construct
  REGION 1..18: note = Synthetic Sequence
DSRATHHRWHYYDNAMDV

SEQ ID NO: 49 - protein, 19 aa, synthetic construct
  REGION 1..19: note = Synthetic Sequence
KAARLSPSRNYSYAYGMDV

SEQ ID NO: 50 - protein, 19 aa, synthetic construct
  REGION 1..19: note = Synthetic Sequence
KAARLSPSMNYSYAYGMDV

SEQ ID NO: 51 - protein, 12 aa, synthetic construct
  REGION 1..12: note = Synthetic Sequence
DLSNRLFTGFDY

SEQ ID NO: 52 - protein, 7 aa, synthetic construct
  REGION 1..7: note = Synthetic Sequence
TFPYFDY

SEQ ID NO: 53 - protein, 8 aa, synthetic construct
  REGION 1..8: note = Synthetic Sequence
RVSLDFDY

SEQ ID NO: 54 - protein, 19 aa, synthetic construct
  REGION 1..19: note = Synthetic Sequence
RYPLLRYAGALYSAYAMDV

SEQ ID NO: 55 - protein, 10 aa, synthetic construct
  REGION 1..10: note = Synthetic Sequence
DTWWEGYFDL

SEQ ID NO: 56 - protein, 7 aa, synthetic construct
  REGION 1..7: note = Synthetic Sequence
VKYIFDY

SEQ ID NO: 57 - protein, 8 aa, synthetic construct
  REGION 1..8: note = Synthetic Sequence
RSQSGFDY

SEQ ID NO: 58 - protein, 7 aa, synthetic construct
  REGION 1..7: note = Synthetic Sequence
CLLQFDY

SEQ ID NO: 59 - protein, 13 aa, synthetic construct
  REGION 1..13: note = Synthetic Sequence
KDVPFKMRFIFDY

SEQ ID NO: 60 - protein, 8 aa, synthetic construct
  REGION 1..8: note = Synthetic Sequence
KIEPDFDY

SEQ ID NO: 61 - protein, 7 aa, synthetic construct
  REGION 1..7: note = Synthetic Sequence
VNHRFDY

SEQ ID NO: 62 - protein, 19 aa, synthetic construct
  REGION 1..19: note = Synthetic Sequence
KGALMCLSATCSSDYGMDV

SEQ ID NO: 63 - protein, 12 aa, synthetic construct
  REGION 1..12: note = Synthetic Sequence
DRSRDMEVDFDY

SEQ ID NO: 64 - protein, 7 aa, synthetic construct
  REGION 1..7: note = Synthetic Sequence
TLTRFDY

SEQ ID NO: 65 - protein, 9 aa, synthetic construct
  REGION 1..9: note = Synthetic Sequence
RDLLYAGDY

SEQ ID NO: 66 - protein, 13 aa, synthetic construct
  REGION 1..13: note = Synthetic Sequence
SGSSSNIGSNDVT

SEQ ID NO: 67 - protein, 13 aa, synthetic construct
  REGION 1..13: note = Synthetic Sequence
TGSSSNIGSNYVS

SEQ ID NO: 68 - protein, 11 aa, synthetic construct
  REGION 1..11: note = Synthetic Sequence
RASQGISNYLA

SEQ ID NO: 69 - protein, 13 aa, synthetic construct
  REGION 1..13: note = Synthetic Sequence
SGSSSNIGSNYVN

SEQ ID NO: 70 - protein, 13 aa, synthetic construct
  REGION 1..13: note = Synthetic Sequence
SGSSSNIGNNAVN

SEQ ID NO: 71 - protein, 13 aa, synthetic construct
  REGION 1..13: note = Synthetic Sequence
TGSSSNIGNNNVT

SEQ ID NO: 72 - protein, 13 aa, synthetic construct
  REGION 1..13: note = Synthetic Sequence
TGSSSNIGNNYVS

SEQ ID NO: 73 - protein, 13 aa, synthetic construct
  REGION 1..13: note = Synthetic Sequence
SGSSSNIGSNSVY

SEQ ID NO: 74 - protein, 13 aa, synthetic construct
  REGION 1..13: note = Synthetic Sequence
SSSSSNIGSNYVN

SEQ ID NO: 75 - protein, 13 aa, synthetic construct
  REGION 1..13: note = Synthetic Sequence
TGSSSNIGNNYVT

SEQ ID NO: 76 - protein, 13 aa, synthetic construct
  REGION 1..13: note = Synthetic Sequence
SGSSSNIGSNTFN

SEQ ID NO: 77 - protein, 13 aa, synthetic construct
  REGION 1..13: note = Synthetic Sequence
SGSSSNIGSNYVS

SEQ ID NO: 78 - protein, 11 aa, synthetic construct
  REGION 1..11: note = Synthetic Sequence
RASQSVSTYLA

SEQ ID NO: 79 - protein, 13 aa, synthetic construct
  REGION 1..13: note = Synthetic Sequence
TGSSSNIGNNTVN

SEQ ID NO: 80 - protein, 13 aa, synthetic construct
  REGION 1..13: note = Synthetic Sequence
SGSSSNIGNNSVT

SEQ ID NO: 81 - protein, 13 aa, synthetic construct
  REGION 1..13: note = Synthetic Sequence
TGSSSNIGSNAVN

SEQ ID NO: 82 - protein, 13 aa, synthetic construct
  REGION 1..13: note = Synthetic Sequence
TGSSSNIGSNTVY

SEQ ID NO: 83 - protein, 13 aa, synthetic construct
  REGION 1..13: note = Synthetic Sequence
TGSSSNIGNNAVS

SEQ ID NO: 84 - protein, 13 aa, synthetic construct
  REGION 1..13: note = Synthetic Sequence
SGSSSNIGSNYVT

SEQ ID NO: 85 - protein, 13 aa, synthetic construct
  REGION 1..13: note = Synthetic Sequence
TGSSSNIGNNNVS

SEQ ID NO: 86 - protein, 13 aa, synthetic construct
  REGION 1..13: note = Synthetic Sequence
SCGGNNIESKAVH

SEQ ID NO: 87 - protein, 7 aa, synthetic construct
  REGION 1..7: note = Synthetic Sequence
DDSKRPS

SEQ ID NO: 88 - protein, 7 aa, synthetic construct
  REGION 1..7: note = Synthetic Sequence
SDSNRPS

SEQ ID NO: 89 - protein, 7 aa, synthetic construct
  REGION 1..7: note = Synthetic Sequence
DASNLES

SEQ ID NO: 90 - protein, 7 aa, synthetic construct
  REGION 1..7: note = Synthetic Sequence
SDSHRPS

SEQ ID NO: 91 - protein, 7 aa, synthetic construct
  REGION 1..7: note = Synthetic Sequence
ADSHRPS

SEQ ID NO: 92 - protein, 7 aa, synthetic construct
  REGION 1..7: note = Synthetic Sequence
SDSQRPS

SEQ ID NO: 93 - protein, 7 aa, synthetic construct
  REGION 1..7: note = Synthetic Sequence
ANSHRPS

SEQ ID NO: 94 - protein, 7 aa, synthetic construct
  REGION 1..7: note = Synthetic Sequence
DNSQRPS

SEQ ID NO: 95 - protein, 7 aa, synthetic construct
  REGION 1..7: note = Synthetic Sequence
DASSLES

SEQ ID NO: 96 - protein, 7 aa, synthetic construct
  REGION 1..7: note = Synthetic Sequence
ADSNRPS

SEQ ID NO: 97 - protein, 7 aa, synthetic construct
  REGION 1..7: note = Synthetic Sequence
YDSHRPS

SEQ ID NO: 98 - protein, 7 aa, synthetic construct
  REGION 1..7: note = Synthetic Sequence
YDNQRPS

SEQ ID NO: 99 - protein, 7 aa, synthetic construct
  REGION 1..7: note = Synthetic Sequence
ADSQRPS

SEQ ID NO: 100 - protein, 7 aa, synthetic construct
  REGION 1..7: note = Synthetic Sequence
SDNQRPS

SEQ ID NO: 101 - protein, 7 aa, synthetic construct
  REGION 1..7: note = Synthetic Sequence
DSSQRPS

SEQ ID NO: 102 - protein, 7 aa, synthetic construct
  REGION 1..7: note = Synthetic Sequence
ANNKRPS

SEQ ID NO: 103 - protein, 11 aa, synthetic construct
  REGION 1..11: note = Synthetic Sequence
AAWDDSLSGYV

SEQ ID NO: 104 - protein, 11 aa, synthetic construct
  REGION 1..11: note = Synthetic Sequence
ATWDASLSAYV

SEQ ID NO: 105 - protein, 9 aa, synthetic construct
  REGION 1..9: note = Synthetic Sequence
QQYANLPYT

SEQ ID NO: 106 - protein, 11 aa, synthetic construct
  REGION 1..11: note = Synthetic Sequence
GSWDSSLNAYV

SEQ ID NO: 107 - protein, 11 aa, synthetic construct
  REGION 1..11: note = Synthetic Sequence
GTWDSSLNGYV

SEQ ID NO: 108 - protein, 11 aa, synthetic construct
  REGION 1..11: note = Synthetic Sequence
GTWDSSLSGYV

SEQ ID NO: 109 - protein, 11 aa, synthetic construct
  REGION 1..11: note = Synthetic Sequence
GTWDYSLNGYV

SEQ ID NO: 110 - protein, 11 aa, synthetic construct
  REGION 1..11: note = Synthetic Sequence
GTWDYSLNAYV

SEQ ID NO: 111 - protein, 11 aa, synthetic construct
  REGION 1..11: note = Synthetic Sequence
GSWDDSLSGYV

SEQ ID NO: 112 - protein, 11 aa, synthetic construct
  REGION 1..11: note = Synthetic Sequence
GTWDDSLNGYV

SEQ ID NO: 113 - protein, 11 aa, synthetic construct
  REGION 1..11: note = Synthetic Sequence
AAWDASLSAYV

SEQ ID NO: 114 - protein, 11 aa, synthetic construct
  REGION 1..11: note = Synthetic Sequence
GAWDSSLNGYV

SEQ ID NO: 115 - protein, 9 aa, synthetic construct
  REGION 1..9: note = Synthetic Sequence
QQSYNLPHT

SEQ ID NO: 116 - protein, 11 aa, synthetic construct
  REGION 1..11: note = Synthetic Sequence
DTWDSSLNAYV

SEQ ID NO: 117 - protein, 11 aa, synthetic construct
  REGION 1..11: note = Synthetic Sequence
ATWDYSLSAYV

SEQ ID NO: 118 - protein, 11 aa, synthetic construct
  REGION 1..11: note = Synthetic Sequence
ASWDASLSGYV

SEQ ID NO: 119 - protein, 11 aa, synthetic construct
  REGION 1..11: note = Synthetic Sequence
GTWEYSLNGYV

SEQ ID NO: 120 - protein, 11 aa, synthetic construct
  REGION 1..11: note = Synthetic Sequence
GTWDYSLSGYV

SEQ ID NO: 121 - protein, 11 aa, synthetic construct
  REGION 1..11: note = Synthetic Sequence
QSYDSNKVVFG

SEQ ID NO: 122 - protein, 121 aa, synthetic construct
  REGION 1..121: note = Synthetic Sequence
EVQLLESGGGLAQPGGSLRLSCAASGFTFSNYDMSWVRQAPGKGPEWVSGIYSGNSNTYYADSVKGRFTISRDNSKNTLYLQMNSLRAEDTAVYYCARDLQYTEWAGFDYWGQGTLVTVSS

SEQ ID NO: 123 - protein, 127 aa, synthetic construct
  REGION 1..127: note = Synthetic Sequence
EVQLLESGGGLVQPGGSLRLSCAASGFTFSDYSMSWVRQAPGKGLEWVSGISHNGGSTYYADSVKGRFTISRDNSKNTLYLQMSSLRAEDTAVYYCARDVSRWSKTRWSYDNAMDVWGQGTLVTVSS

SEQ ID NO: 124 - protein, 121 aa, synthetic construct
  REGION 1..121: note = Synthetic Sequence
EVQLLESGGGLVQPGGSLRLSCAASGFTFSSYAMSWVRQAPGKGLEWVSGISPGGSSKYYADSVKGRFTISRDNSKNTLYLQMNSLRAEDTAVYYCARGPHRAIDTAFDYWGQGTLVTVSS

SEQ ID NO: 125 - protein, 119 aa, synthetic construct
  REGION 1..119: note = Synthetic Sequence
EVQLLESGGGLVQPGGSLRLSCAASGFTFSDYAMAWVRQAPGKGLEWVSIIYPGDSETIYSPSFEGRFTISRDNSKNTLYLQMNSLRAEDTAVYYCARDTYWEGYFDLWGQGTLVTVSS

SEQ ID NO: 126 - protein, 127 aa, synthetic construct; identical to SEQ ID NO: 123
  REGION 1..127: note = Synthetic Sequence

SEQ ID NO: 127 - protein, 127 aa, synthetic construct
  REGION 1..127: note = Synthetic Sequence
EVQLLESGGGLVQPGGSLRLSCAASGFTFSNYSMSWVRQAPGKGLEWVSAISHGSGSIYYADSVKGRFTISRDNSKNTLYLQMNSLRAEDTAVYYCAKPISAWSHIRMSYAYGMDVWGQGTLVTVSS

SEQ ID NO: 128 - protein, 127 aa, synthetic construct
  REGION 1..127: note = Synthetic Sequence
EVQLLESGGGLVQPGGSLRLSCAASGFTFSGYSMSWVRQAPGKGLEWVSGISYGGSSISYADSVKGRFTISRDNSKNTLYLQMNSLRAEDTAVYYCAKPVRRWARFRLSYDDAMDVWGQGTLVTVSS

SEQ ID NO: 129 - protein, 127 aa, synthetic construct
  REGION 1..127: note = Synthetic Sequence
EVQLLESGGGLVQPGGSLRLSCAASGFTFSNYSMSWVRQAPGKGLEWVSGIYSGNSNTYYADSVKGRFTISRDNSKNTLYLQMNSLRAEDTAVYYCAKDSRATHHRWHYYDNAMDVWGQGTLVTVSS

SEQ ID NO: 130 - protein, 127 aa, synthetic construct
  REGION 1..127: note = Synthetic Sequence
EVQLLESGGGLVQPGGSLRLSCAASGFTFSNYAMSWVRQAPGKGLEWVSGISPNGSSIYYADSVKGRFTISRDNSKNTLYLQMNSLRAEDTAVYYCAKAARLSPSRNYSYAYGMDVWGQGTLVTVSS

SEQ ID NO: 131 - protein, 127 aa, synthetic construct
  REGION 1..127: note = Synthetic Sequence
EVQLLESGGGLVQPGGSLRLSCAASGFTFSNYAMSWVRQAPGKGLEWVSGISPDGGSIYYADSVKGRFTISRDNSKNTLYLQMNSLRAEDTAVYYCAKAARLSPSMNYSYAYGMDVWGQGTLVTVSS

SEQ ID NO: 132 - protein, 127 aa, synthetic construct; identical to SEQ ID NO: 128
  REGION 1..127: note = Synthetic Sequence

SEQ ID NO: 133 - protein, 121 aa, synthetic construct
  REGION 1..121: note = Synthetic Sequence
EVQLLESGGGLVQPGGSLRLSCAASGFTFSSYDMSWVRQVPGKGLEWVSWISHGGGSIYYADSVKGRFTISRDNSKNTLYLQMNSLRAEDTAVYYCARDLSNRLFTGFDYWGQGTLVAVSS

SEQ ID NO: 134 - protein, 116 aa, synthetic construct
  REGION 1..116: note = Synthetic Sequence
EVQLLESGGGLVQPGGSLRLSCAVSGFTFSSYSMSWVRQAPGKGLEWVSAISPGDSNKYYADSVKGRFTISRDNSKNTLYLQINSLRAEDTAVYYCARTFPYFDYWGQGTLVTVSS

SEQ ID NO: 135 - protein, 127 aa, synthetic construct
  REGION 1..127: note = Synthetic Sequence
EVQLLESGGGLVQPGGSLRLSCAASGFTFSNYAMSWVRQAPGKGLEWVSGISPGGGSIYYADSVKGRFTISRDNSKNTLYLQMNSLRAEDTAVYYCAKAARLSPSMNYSYAYGMDVWGQGTLVTVSS

SEQ ID NO: 136 - protein, 116 aa, synthetic construct
  REGION 1..116: note = Synthetic Sequence
EVQLLESGGGLVQTGGSLRLSCAASGFTFSDYAMSWVRQAPGKGLEWVSAISHGGSSKYYADSVKGRFTISRDNSKNTLYLQMNSLRAEDTAVYYCARVSLDFDYWGQGTLVAVSS

SEQ ID NO: 137 - protein, 127 aa, synthetic construct
  REGION 1..127: note = Synthetic Sequence
EVQLLESGGGLVQPGGSLRLSCAASGFTFSGYAMSWVRQAPGKGLEWVSVISPGSGSKYYADSVRGRFTVSRDNSKNTLYLQMNSLRAEDTAVYYCARYPLLRYAGALYSAYAMDVWGQGTLVTVSS

SEQ ID NO: 138 - protein, 118 aa, synthetic construct
  REGION 1..118: note = Synthetic Sequence
EVQLLESGGGLVQPDGSMRLICAASGFTFSSYAKHWVRQAPGKGLEWVSEIYTSGSTNYNPSLKSRFTISRDNSKNTLYLQMNSLRAEDTAVYYCARDTWWEGYFDLWGQGTLVTVSS

SEQ ID NO: 139 - protein, 116 aa, synthetic construct
  REGION 1..116: note = Synthetic Sequence
EVQLLESGGGLVQPGGSLRLSCAASGFTFSGYYMSWVRQAPGKGLEWVSVISHDGSSTYYADSVKGRFTISRDNSKNTLYLQMNSLRAEDTAVYYCAKVKYIFDYWGQGTLVTVSS

SEQ ID NO: 140 - protein, 116 aa, synthetic construct
  REGION 1..116: note = Synthetic Sequence
EVQLLESGGGLVQPGGSLRLSCAASGFTFSSYAMSWVRQAPGKGLEWVSWISPGGGNIYYADSVKGRFTISRDNSKNTLYLQMNSLRAEDTAVYYCARSQSGFDYWGQGTLVTVSS

SEQ ID NO: 141 - protein, 116 aa, synthetic construct
  REGION 1..116: note = Synthetic Sequence
EVQLLESGGGLVQPGGSLRLSCAASGFTFSNYDMSWVRQAPGKGLEWVSSISSNGGSTYYADSVKGRFTISRDNSKNTLYLQMNSLRAEDTAVYYCAKCLLQFDYWGQGTLVTVSS

SEQ ID NO: 142 - protein, 121 aa, synthetic construct
  REGION 1..121: note = Synthetic Sequence
EVQLLESGGGLVQPGGSLRLSCAASGFTFSGYDMSWVRQAPGKGLEWVSGISHDGRSKYYADSVKGRFTVSRDNSKNTLYLQMNSLRAEDTAVYYCAKDVPFKMRFIFDYWGQGTLVTVSS

SEQ ID NO: 143 - protein, 116 aa, synthetic construct
  REGION 1..116: note = Synthetic Sequence
EVQLLESGGGLVQPGGSLRLSCAASGFTFSDYYMSWVRQAPGKGLEWVSLISPGSDSKYYADSVKGRFTISRDNSKNTLYLQMNSLRAEDTAVYYCAKIEPDFDYWGQGTLVTVSS

SEQ ID NO: 144 - protein, 116 aa, synthetic construct
  REGION 1..116: note = Synthetic Sequence
EVQLLESGGGMVQTGGSLRLSCAASGFTFSDYAMSWVRQAPGKGLEWVSAISYDNGNTYYADSVKGRFTISRDNSKNALYLQMNSLRAEDTAVYYCAKVNHRFDYWGQGTLVTVSS

SEQ ID NO: 145 - protein, 127 aa, synthetic construct
  REGION 1..127: note = Synthetic Sequence
EVQLQESGGGLVLPGGSLRLSCAASGFTFNNYAMSWVRQAPGKGLEWVSGISPNGSSIYYADSVKGRFTISRDNSKNTLYLQMNSLRAEDTAVYYCAKAARLSPSRNYSYAYGMDVWGQGTLVTVSS

SEQ ID NO: 146 - protein, 127 aa, synthetic construct
  REGION 1..127: note = Synthetic Sequence
EVQLLESGGGLVQPGGSLRLSCAASGFTFSDYAMSWVRQAPGKGLEWVSWISPGGGNTYYADSVKGRFTISRDNSKNTLYLQMNSLRAEDTAVYYCAKGALMCLSATCSSDYGMDVWGQGTLVTVSS

SEQ ID NO: 147 - protein, 127 aa, synthetic construct; identical to SEQ ID NO: 130
  REGION 1..127: note = Synthetic Sequence

SEQ ID NO: 148 - protein, 127 aa, synthetic construct; identical to SEQ ID NO: 130
  REGION 1..127: note = Synthetic Sequence

SEQ ID NO: 149 - protein, 121 aa, synthetic construct
  REGION 1..121: note = Synthetic Sequence
EVQLLESGGGLVQPGGSLRLSCAASGFTFSDYAMSWVRQAPGKGLEWVSVISSDGGSIYYADSVKGRFTISRDNSKNTLYLQMNSLRAEDTAVYYCAKDRSRDMEVDFDYWGQGTLVTVSS

SEQ ID NO: 150 - protein, 121 aa, synthetic construct; identical to SEQ ID NO: 149
  REGION 1..121: note = Synthetic Sequence

SEQ ID NO: 151 - protein, 116 aa, synthetic construct
  REGION 1..116: note = Synthetic Sequence
EVQLLESGGGLVQPGGSLRLSCAASGFTFSNYDMSWVRQAPGKGLEWVSWISPGGSSIYYADSVKGRFTISRDNSKNTLYLQMNSLRAEDTAVYYCAKTLTRFDYWGQGTLVTVSS

SEQ ID NO: 152 - protein, 116 aa, synthetic construct
  REGION 1..116: note = Synthetic Sequence
EVQLLESGGGLVQPGGSLRLSCAASGFTFSNYAMHWVRQAPGKGLEWVSIIYPDDDTRYNPSFRGRFTISRDNSKNTLYLQMNSLRAEDTAVYYCARDLLYAGDYWGQGTLVTVSS

SEQ ID NO: 153 - protein, 110 aa, synthetic construct
  REGION 1..110: note = Synthetic Sequence
QSVLTQPPSASGTPGQRVTISCSGSSSNIGSNDVTWYQQLPGTAPKLLIYDDSKRPSGVPDRFSGSKSGTSASLAISGLRSEDEADYYCAAWDDSLSGYVFGGGTKLTVL

SEQ ID NO: 154 - protein, 110 aa, synthetic construct
  REGION 1..110: note = Synthetic Sequence
QSVLTQPPSASGTPGQRVTISCTGSSSNIGSNYVSWYRQLPGTAPKLLIYSDSNRPSGVPDRFSGSKSGTSASLAISGLRSEDEADYYCATWDASLSAYVFGGGTKLTVL

SEQ ID NO: 155 - protein, 110 aa, synthetic construct; identical to SEQ ID NO: 154
  REGION 1..110: note = Synthetic Sequence

SEQ ID NO: 156 - protein, 107 aa, synthetic construct
  REGION 1..107: note = Synthetic Sequence
EIVLTQSPGTLSLSPGERATLSCRASQGISNYLAWYQQKPGQAPRLLIYDASNLESGIPDRFSGSGSGTDFTLTISRLEPEDFAVYYCQQYANLPYTFGQGTKVEIK

SEQ ID NO: 157 - protein, 110 aa, synthetic construct
  REGION 1..110: note = Synthetic Sequence
QSVLTQPPSASGTPGQRVTISCSGSSSNIGSNYVNWYQQLPGTAPKLLIYSDSHRPSGVPDRFSGSKSGTSASLAISGLRSEDEADYYCGSWDSSLNAYVLGGGTKLTVL

SEQ ID NO: 158 - protein, 110 aa, synthetic construct; identical to SEQ ID NO: 154
  REGION 1..110: note = Synthetic Sequence

SEQ ID NO: 159 - protein, 110 aa, synthetic construct
  REGION 1..110: note = Synthetic Sequence
QSVLTQPPSASGTPGQRVTISCSGSSSNIGNNAVNWYQQLPGTAPKLLIYADSHRPSGVPDRFSGSKSGTSASLAISGLRSEDEADYYCGTWDSSLNGYVFGGGTKLTVL

SEQ ID NO: 160 - protein, 110 aa, synthetic construct
  REGION 1..110: note = Synthetic Sequence
QSVLTQPPSASGTPGQRVTISCTGSSSNIGSNYVSWYRQLPGTAPKLLIYSDSNRPSGVPDRFSGSKSGTSASLAISGLRSEDEADYYCGTWDSSLSGYVFGGGTKLTVL

SEQ ID NO: 161 - protein, 110 aa, synthetic construct
  REGION 1..110: note = Synthetic Sequence
QSVLTQPPSASGTPGQRVTISCTGSSSNIGNNNVTWYQQLPGTAPKLLIYSDSQRPSGVPDRFSGSKSGTSASLAISGLRSEDEADYYCGTWDYSLNGYVFGGGTKLTVL

SEQ ID NO: 162 - protein, 110 aa, synthetic construct
  REGION 1..110: note = Synthetic Sequence
QSVLTQPPSASGTPGQRVTISCTGSSSNIGNNYVSWYQQLPGTAPKLLIYSDSHRPSGVPDRFSGSKSGTSASLAISGLRSEDEADYYCGTWDYSLNGYVFGGGTKLTVL

SEQ ID NO: 163 - protein, 110 aa, synthetic construct
  REGION 1..110: note = Synthetic Sequence
QSVLTQPPSASGTPGQRVTISCSGSSSNIGNNAVNWYQQLPGTAPKLLIYANSHRPSGVPDRFSGSKSGTSASLAISGLRSEDEADYYCGTWDSSLSGYVFGGGTKLTVL

SEQ ID NO: 164 - protein, 110 aa, synthetic construct
  REGION 1..110: note = Synthetic Sequence
QSVLTQPPSASGTPGQRVTISCSGSSSNIGSNSVYWYQQLPGTAPKPLIYSDSHRPSGVPDRFSGSKSGTSASLAISGLRSEDEADYYCGTWDYSLNAYVFGGGTKLTVL

SEQ ID NO: 165 - protein, 110 aa, synthetic construct
  REGION 1..110: note = Synthetic Sequence
QSVLTQPPSASGTPGERVTISCSSSSSNIGSNYVNWYQQLPGTAPKLLIYDNSQRPSGVPDRFSGSKSGTSASLAISGLRSEDEADYYCGSWDDSLSGYVFGGGTKLTVL

SEQ ID NO: 166 - protein, 110 aa, synthetic construct
  REGION 1..110: note = Synthetic Sequence
QSVLTQPPSASGTPGQRVTISCTGSSSNIGNNYVTWYQQLPGTAPRLLIYSDSQRPSGVPDRFSGSKSGTSASLAISGLRSEDEADYYCGTWDDSLNGYVFGGGTKLTVL

SEQ ID NO: 167 - protein, 110 aa, synthetic construct
  REGION 1..110: note = Synthetic Sequence
QSVLTQPPSASGTPGQRVTISCSGSSSNIGSNTFNWYQQLPGTAPKLLIYADSHRPSGVPDRFSGSKSGTSASLAISGLRSEDEADYYCAAWDASLSAYVFGGGTKLTVL

SEQ ID NO: 168 - protein, 110 aa, synthetic construct
  REGION 1..110: note = Synthetic Sequence
QSVLTQPPSASGTPGQRVTISCSGSSSNIGSNYVSWYQQLPGTAPKLLIYANSHRPSGVPDRFSGSKSGTSASLAISGLRSEDEADYYCGAWDSSLNGYVFGGGTKLTVL

SEQ ID NO: 169 - protein, 107 aa, synthetic construct
  REGION 1..107: note = Synthetic Sequence
EIVLTQSPGTLSLSPGERATLSCRASQSVSTYLAWYQQKPGQAPRLLIYDASSLESGIPDRFSGSGSGTDFTLTISRLEPEDFAVYYCQQSYNLPHTFGQGTKVEIK

SEQ ID NO: 170 - protein, 110 aa, synthetic construct
  REGION 1..110: note = Synthetic Sequence
QSVLTQPPSASGTPGQRVTISCTGSSSNIGNNTVNWYQQLPGTAPKLLIYADSNRPSGVPDRFSGSKSGTSASLAISGLRSEDEADYYCDTWDSSLNAYVFGGGTKLTVL

SEQ ID NO: 171 - protein, 110 aa, synthetic construct
  REGION 1..110: note = Synthetic Sequence
QSVLTQPPSASGTPGQRVTISCSGSSSNIGNNSVTWYQQLPGTAPKLLIYYDSHRPSGVPDRFSGSKSGTSASLAISGLRSEDEADYYCGAWDSSLNGYVFGGGTKLTVL

SEQ ID NO: 172 - protein, 110 aa, synthetic construct
  REGION 1..110: note = Synthetic Sequence
QSVLTQPPSASGTPGQRVTISCTGSSSNIGSNAVNWYQQLPGTAPKLLIYYDNQRPSGVPDRFSGSKSGTSASLAISGLRSEDEADYYCAAWDDSLSGYVFGGGTKLTVL

SEQ ID NO: 173 - protein, 110 aa, synthetic construct
  REGION 1..110: note = Synthetic Sequence
QSVLTQPPSASGTPGQRVTLSCTGSSSNIGSNTVYWYQQLPGTAPKLLIYADSQRPSGVPDRFSGSKSGTSASLAISGLRSEDEADYYCGSWDSSLNAYVFGGGTKLTVL

SEQ ID NO: 174 - protein, 110 aa, synthetic construct
  REGION 1..110: note = Synthetic Sequence
QSVLTQPPSASGTPGQRVTISCSGSSSNIGSNTFNWYQQLPGTAPKLLIYADSHRPSGVPDRFSGSKSGTSASLAISGLRSEDEADYYCATWDYSLSAYVFGGGTKLTVL

SEQ ID NO: 175 - protein, 110 aa, synthetic construct
  REGION 1..110: note = Synthetic Sequence
QSVLTQPPSASGTPGQRVTISCSGSSSNIGSNTFNWYQQLPGTAPKLLIYANSHRPSGVPDRFSGSKSGTSASLAISGLRSEDEADYYCASWDASLSGYVFGGGTKLTVL

SEQ ID NO: 176 - protein, 110 aa, synthetic construct; identical to SEQ ID NO: 161
  REGION 1..110: note = Synthetic Sequence

SEQ ID NO: 177 - protein, 110 aa, synthetic construct
  REGION 1..110: note = Synthetic Sequence
QSVLTQPPSASGTPGQRVTISCTGSSSNIGNNAVSWYQQLPGTAPKLLIYSDNQRPSGVPDRFSGSKSGTSASLAISGLRSEDEADYYCGTWDYSLNGYVFGGGTKLTVL

SEQ ID NO: 178 - protein, 110 aa, synthetic construct
  REGION 1..110: note = Synthetic Sequence
QSVLTQPPSASGTPGQRVTISCTGSSSNIGNNNVTWYQQLPGTAPKLLIYSDSQRPSGVPDRFSGSKSGTSASLAISGLRSKDEADYYCGTWDYSLNGYVFGGGTKLTVL

SEQ ID NO: 179 - protein, 110 aa, synthetic construct
  REGION 1..110: note = Synthetic Sequence
QSVLTQPPSASGTPGQRVTISCTGSSSNIGNNNVTWYQQLPGTAPKLLIYSDSQRPSGVPDRFSGSKSGTSASLAISGLRSEDEADYYCGTWEYSLNGYVFGGGTKLTVL

SEQ ID NO: 180 - protein, 110 aa, synthetic construct
  REGION 1..110: note = Synthetic Sequence
QSVLTQPPSASGTPGQRVTISCSGSSSNIGSNYVTWYQQLPGTAPKLLIYDSSQRPSGVPDRFSGSKSGTSASLAISGLRSEDEADYYCGTWDYSLSGYVFGGGTKLTVL

SEQ ID NO: 181 - protein, 110 aa, synthetic construct
  REGION 1..110: note = Synthetic Sequence
QSVLTQPPSASGTPGQRVTISCSGSSSNIGSNYVTWYQQLPGTAPKLLIYDSSQRPSGVPDRFSGSKSGTSASLAISGLRSEDEADYYCGTWDYSLNGYVFGGGTKLTVL

SEQ ID NO: 182 - protein, 110 aa, synthetic construct
  REGION 1..110: note = Synthetic Sequence
QSVLTQPPSASGTPGQRVTISCTGSSSNIGNNNVSWYQQLPGTAPKLLIYYDSHRPSGVPDRFSGSKSGTSASLAISGLRSEDEADYYCGTWDSSLSGYVFGGGTKLTVL

SEQ ID NO: 183 - protein, 106 aa, synthetic construct
  REGION 1..106: note = Synthetic Sequence
QSVLTQPPSASGTPGQRVTISCGGNNIESKAVHWYQQLPGTAPKLLIYANNKRPSGVPDRFSGSKSGTSASLAISGLRSEDEADYYCQSYDSNKVVFGGGTKLTVL

SEQ ID NO: 184 - protein, 17 aa, synthetic construct
VISSDVGSIYYADSVKG

SEQ ID NO: 185 - protein, 17 aa, synthetic construct
VISSDKGSIYYADSVKG

SEQ ID NO: 186 - protein, 7 aa, synthetic construct
DASQRPS

SEQ ID NO: 187 - protein, 7 aa, synthetic construct
DKSQRPS

SEQ ID NO: 188 - protein, 121 aa, synthetic construct
EVQLLESGGGLVQPGGSLRLSCAASGFTFSDYAMSWVRQAPGKGLEWVSVISSDVGSIYYADSVKGRFTISRDNSKNTLYLQMNSLRAEDTAVYYCAKDRSRDMEVDFDYWGQGTLVTVSS

SEQ ID NO: 189 - protein, 121 aa, synthetic construct
EVQLLESGGGLVQPGGSLRLSCAASGFTFSDYAMSWVRQAPGKGLEWVSVISSDKGSIYYADSVKGRFTISRDNSKNTLYLQMNSLRAEDTAVYYCAKDRSRDMEVDFDYWGQGTLVTVSS

SEQ ID NO: 190 - protein, 121 aa, synthetic construct; identical to SEQ ID NO: 149

SEQ ID NO: 191 - protein, 121 aa, synthetic construct; identical to SEQ ID NO: 149

SEQ ID NO: 192 - protein, 121 aa, synthetic construct; identical to SEQ ID NO: 149

SEQ ID NO: 193 - protein, 121 aa, synthetic construct; identical to SEQ ID NO: 189

SEQ ID NO: 194 - protein, 110 aa, synthetic construct; identical to SEQ ID NO: 181

SEQ ID NO: 195 - protein, 110 aa, synthetic construct; identical to SEQ ID NO: 181

SEQ ID NO: 196 - protein, 110 aa, synthetic construct
QSVLTQPPSASGTPGQRVTISCSGSSSNIGSNYVTWYQQLPGTAPKLLIYDASQRPSGVPDRFSGSKSGTSASLAISGLRSEDEADYYCGTWDYSLNGYVFGGGTKLTVL

SEQ ID NO: 197 - protein, 110 aa, synthetic construct
QSVLTQPPSASGTPGQRVTISCSGSSSNIGSNYVTWYQQLPGTAPKLLIYDKSQRPSGVPDRFSGSKSGTSASLAISGLRSEDEADYYCGTWDYSLNGYVFGGGTKLTVL

SEQ ID NO: 198 - protein, 110 aa, synthetic construct
QSVLTQPPSASGTPGQRVTISCSGSSSNIGSNYVTWYQQLPGTAPKLLIYDSSQRPSGVPDRFSGSKSGTSASLAISGLRSEDEADYYCGTWDYSLNAYVFGGGTKLTVL

SEQ ID NO: 199 - protein, 110 aa, synthetic construct
QSVLTQPPSASGTPGQRVTISCSGSSSNIGSNYVTWYQQLPGTAPKLLIYDKSQRPSGVPDRFSGSKSGTSASLAISGLRSEDEADYYCGTWDYSLNAYVFGGGTKLTVL

SEQ ID NO: 200 - protein, 15 aa, synthetic construct
GGGGSGGGGSGGGGS